European Patent Application EP 4 512 421 A1, published February 26, 2025. Title: Drug combination of anti-TIM-3 antibody and anti-PD-1 antibody. Applicant: Nanjing Shunxin Pharmaceuticals Co.,LTD. of Chiatai Tianqing Pharmaceutical Group. Application EP EP23803036.5, filed May 12, 2023. The sequence listing filed with the application follows.

SEQUENCE LISTING (31 sequences)

SEQ ID NO: 1 - protein, 10 aa, synthetic construct
  source 1..10: note = HCDR1 of anti-TIM-3 antibody
GYSFTGYTIN

SEQ ID NO: 2 - protein, 10 aa, synthetic construct
  source 1..10: note = HCDR2 of anti-TIM-3 antibody
LFNPYNGGTT

SEQ ID NO: 3 - protein, 10 aa, synthetic construct
  source 1..10: note = HCDR3 of anti-TIM-3 antibody
RYYGYDAMDY

SEQ ID NO: 4 - protein, 17 aa, synthetic construct
  source 1..17: note = LCDR1 of anti-TIM-3 antibody
KSSQSVLYSSNQKNHLA

SEQ ID NO: 5 - protein, 7 aa, synthetic construct
  source 1..7: note = LCDR2 of anti-TIM-3 antibody
WASTRES

SEQ ID NO: 6 - protein, 8 aa, synthetic construct
  source 1..8: note = LCDR3 of anti-TIM-3 antibody
HQYLSSYT

SEQ ID NO: 7 - protein, 119 aa, synthetic construct
  source 1..119: note = VH of anti-TIM-3 antibody
QVQLVQSGAEVKKPGASVKVSCKASGYSFTGYTINWVRQAPGQGLEWMGLFNPYNGGTTYAQKFQGRVTMTVDKSTSTVYMELSSLRSEDTAVYYCARRYYGYDAMDYWGQGTLVTVSS

SEQ ID NO: 8 - protein, 112 aa, synthetic construct
  source 1..112: note = VL of anti-TIM-3 antibody
DIQMTQSPSSLSASVGDRVTITCKSSQSVLYSSNQKNHLAWYQQKPGKAPKLLIYWASTRESGVPSRFSGSGSGTDFTLTISSLQPEDFATYYCHQYLSSYTFGQGTKLEIK

SEQ ID NO: 9 - protein, 446 aa, synthetic construct
  source 1..446: note = Heavy chain of anti-TIM-3 antibody
QVQLVQSGAEVKKPGASVKVSCKASGYSFTGYTINWVRQAPGQGLEWMGLFNPYNGGTTYAQKFQGRVTMTVDKSTSTVYMELSSLRSEDTAVYYCARRYYGYDAMDYWGQGTLVTVSSASTKGPSVFPLAPCSRSTSESTAALGCLVKDYFPEPVTVSWNSGALTSGVHTFPAVLQSSGLYSLSSVVTVPSSSLGTKTYTCNVDHKPSNTKVDKRVESKYGPPCPPCPAPEFLGGPSVFLFPPKPKDTLMISRTPEVTCVVVDVSQEDPEVQFNWYVDGVEVHNAKTKPREEQFNSTYRVVSVLTVLHQDWLNGKEYKCKVSNKGLPSSIEKTISKAKGQPREPQVYTLPPSQEEMTKNQVSLTCLVKGFYPSDIAVEWESNGQPENNYKTTPPVLDSDGSFFLYSRLTVDKSRWQEGNVFSCSVMHEALHNHYTQKSLSLSLGK

SEQ ID NO: 10 - protein, 219 aa, synthetic construct
  source 1..219: note = Light chain of anti-TIM-3 antibody
DIQMTQSPSSLSASVGDRVTITCKSSQSVLYSSNQKNHLAWYQQKPGKAPKLLIYWASTRESGVPSRFSGSGSGTDFTLTISSLQPEDFATYYCHQYLSSYTFGQGTKLEIKRTVAAPSVFIFPPSDEQLKSGTASVVCLLNNFYPREAKVQWKVDNALQSGNSQESVTEQDSKDSTYSLSSTLTLSKADYEKHKVYACEVTHQGLSSPVTKSFNRGEC

SEQ ID NO: 11 - protein, 8 aa, synthetic construct
  source 1..8: note = HCDR1 of anti-PD-1 antibody
GFAFSSYD

SEQ ID NO: 12 - protein, 8 aa, synthetic construct
  source 1..8: note = HCDR2 of anti-PD-1 antibody
ISGGGRYT

SEQ ID NO: 13 - protein, 11 aa, synthetic construct
  source 1..11: note = HCDR3 of anti-PD-1 antibody
ANRYGEAWFAY

SEQ ID NO: 14 - protein, 6 aa, synthetic construct
  source 1..6: note = LCDR1 of anti-PD-1 antibody
QDINTY

SEQ ID NO: 15 - skipped

SEQ ID NO: 16 - protein, 9 aa, synthetic construct
  source 1..9: note = LCDR3 of anti-PD-1 antibody
LQYDEFPLT

SEQ ID NO: 17 - protein, 118 aa, synthetic construct
  source 1..118: note = VH of anti-PD-1 antibody
EVQLVESGGGLVQPGGSLRLSCAASGFAFSSYDMSWVRQAPGKGLDWVATISGGGRYTYYPDSVKGRFTISRDNSKNNLYLQMNSLRAEDTALYYCANRYGEAWFAYWGQGTLVTVSS

SEQ ID NO: 18 - protein, 107 aa, synthetic construct
  source 1..107: note = VL of anti-PD-1 antibody
DIQMTQSPSSMSASVGDRVTFTCRASQDINTYLSWFQQKPGKSPKTLIYRANRLVSGVPSRFSGSGSGQDYTLTISSLQPEDMATYYCLQYDEFPLTFGAGTKLELK

SEQ ID NO: 19 - protein, 448 aa, synthetic construct
  source 1..448: note = Heavy chain of anti-PD-1 antibody
EVQLVESGGGLVQPGGSLRLSCAASGFAFSSYDMSWVRQAPGKGLDWVATISGGGRYTYYPDSVKGRFTISRDNSKNNLYLQMNSLRAEDTALYYCANRYGEAWFAYWGQGTLVTVSSASTKGPSVFPLAPSSKSTSGGTAALGCLVKDYFPEPVTVSWNSGALTSGVHTFPAVLQSSGLYSLSSVVTVPSSSLGTQTYICNVNHKPSNTKVDKKVEPKSCDKTHTCPPCPAPEAAGAPSVFLFPPKPKDTLMISRTPEVTCVVVDVSHEDPEVKFNWYVDGVEVHNAKTKPREEQYNSTYRVVSVLTVLHQDWLNGKEYKCKVSNKALPAPIEKTISKAKGQPREPQVYTLPPSRDELTKNQVSLTCLVKGFYPSDIAVEWESNGQPENNYKTTPPVLDSDGSFFLYSKLTVDKSRWQQGNVFSCSVMHEALHNHYTQKSLSLSPGK

SEQ ID NO: 20 - protein, 214 aa, synthetic construct
  source 1..214: note = Light chain of anti-PD-1 antibody
DIQMTQSPSSMSASVGDRVTFTCRASQDINTYLSWFQQKPGKSPKTLIYRANRLVSGVPSRFSGSGSGQDYTLTISSLQPEDMATYYCLQYDEFPLTFGAGTKLELKRTVAAPSVFIFPPSDEQLKSGTASVVCLLNNFYPREAKVQWKVDNALQSGNSQESVTEQDSKDSTYSLSSTLTLSKADYEKHKVYACEVTHQGLSSPVTKSFNRGEC

SEQ ID NO: 21 - protein, 10 aa, synthetic construct
  source 1..10: note = HCDR1 of another anti-TIM-3 antibody
GFNIKDYYMH

SEQ ID NO: 22 - protein, 11 aa, synthetic construct
  source 1..11: note = HCDR2 of another anti-TIM-3 antibody
WIDPENDNTIY

SEQ ID NO: 23 - protein, 12 aa, synthetic construct
  source 1..12: note = HCDR3 of another anti-TIM-3 antibody
ARDFGYVAWLVY

SEQ ID NO: 24 - protein, 11 aa, synthetic construct
  source 1..11: note = LCDR1 of another anti-TIM-3 antibody
KASQNVDTAVA

SEQ ID NO: 25 - protein, 7 aa, synthetic construct
  source 1..7: note = LCDR2 of another anti-TIM-3 antibody
SASNRYT

SEQ ID NO: 26 - protein, 8 aa, synthetic construct
  source 1..8: note = LCDR3 of another anti-TIM-3 antibody
QQYSSYPT

SEQ ID NO: 27 - protein, 119 aa, synthetic construct
  source 1..119: note = VH of another anti-TIM-3 antibody
EVQLQQSGAEVVRPGALVKLSCKASGFNIKDYYMHWVRQRPEQGLEWIGWIDPENDNTIYDPKFQDRASITADTSSNTAYLQLSSLTSEDTAVYYCARDFGYVAWLVYWGQGTLVTVSA

SEQ ID NO: 28 - protein, 106 aa, synthetic construct
  source 1..106: note = VL of another anti-TIM-3 antibody
DIVMTQSQEFMSTSVGDRVSITCKASQNVDTAVAWYQQKPGQSPKLLIYSASNRYTGVPDRFTGTGSGTDFTLTINNMQSEDLADYFCQQYSSYPTFGGRTKLEIK

SEQ ID NO: 29 - protein, 446 aa, synthetic construct
  source 1..446: note = Heavy chain of another anti-TIM-3 antibody
EVQLQQSGAEVVRPGALVKLSCKASGFNIKDYYMHWVRQRPEQGLEWIGWIDPENDNTIYDPKFQDRASITADTSSNTAYLQLSSLTSEDTAVYYCARDFGYVAWLVYWGQGTLVTVSAASTKGPSVFPLAPCSRSTSESTAALGCLVKDYFPEPVTVSWNSGALTSGVHTFPAVLQSSGLYSLSSVVTVPSSSLGTKTYTCNVDHKPSNTKVDKRVESKYGPPCPPCPAPEFLGGPSVFLFPPKPKDTLMISRTPEVTCVVVDVSQEDPEVQFNWYVDGVEVHNAKTKPREEQFNSTYRVVSVLTVLHQDWLNGKEYKCKVSNKGLPSSIEKTISKAKGQPREPQVYTLPPSQEEMTKNQVSLTCLVKGFYPSDIAVEWESNGQPENNYKTTPPVLDSDGSFFLYSRLTVDKSRWQEGNVFSCSVMHEALHNHYTQKSLSLSLGK

SEQ ID NO: 30 - protein, 213 aa, synthetic construct
  source 1..213: note = Light chain of another anti-TIM-3 antibody
DIVMTQSQEFMSTSVGDRVSITCKASQNVDTAVAWYQQKPGQSPKLLIYSASNRYTGVPDRFTGTGSGTDFTLTINNMQSEDLADYFCQQYSSYPTFGGRTKLEIKRTVAAPSVFIFPPSDEQLKSGTASVVCLLNNFYPREAKVQWKVDNALQSGNSQESVTEQDSKDSTYSLSSTLTLSKADYEKHKVYACEVTHQGLSSPVTKSFNRGEC

SEQ ID NO: 31 - protein, 12 aa, synthetic construct
  source 1..12: note = HCDR3 of anti-TIM-3 antibody
ARRYYGYDAMDY